European Patent Specification EP 3 899 053 B1, published January 10, 2024. Title: COMPOSITIONS AND METHODS FOR DETECTING PLASMODIUM SPECIES NUCLEIC ACID. Applicant: Gen-Probe Incorporated Grifols Diagnostic Solutions Inc. SELF, Deanna LINNEN, Jeffrey M. BRES, Vanessa. The sequence listing filed with the application follows.

SEQUENCE LISTING (197 sequences)

SEQ ID NO: 1 - DNA, 55 bp, Artificial Sequence
  Synthetic Oligonucleotide
  misc_feature (23)..(55)
ggauuggguaauuugcgcgccctttaaaaaaaaaaaaaaaaaaaaaaaaaaaaaa

SEQ ID NO: 2 - DNA, 61 bp, Artificial Sequence
  Synthetic Oligonucleotide
  misc_feature (29)..(61)
caagaaagagcuaucaaucugucaaucctttaaaaaaaaaaaaaaaaaaaaaaaaaaaaaa

SEQ ID NO: 3 - DNA, 59 bp, Artificial Sequence
  Synthetic Oligonucleotide
  misc_feature (27)..(59)
cccguguugagucaaauuaagccgcatttaaaaaaaaaaaaaaaaaaaaaaaaaaaaaa

SEQ ID NO: 4 - DNA, 55 bp, Artificial Sequence
  Synthetic Oligonucleotide
  misc_feature (23)..(55)
ggguaauuugcgcgccugcugctttaaaaaaaaaaaaaaaaaaaaaaaaaaaaaa

SEQ ID NO: 5 - DNA, 59 bp, Artificial Sequence
  Synthetic Oligonucleotide
  misc_feature (27)..(59)
uuucucaggcucccucuccggaaucgtttaaaaaaaaaaaaaaaaaaaaaaaaaaaaaa

SEQ ID NO: 6 - DNA, 57 bp, Artificial Sequence
  Synthetic Oligonucleotide
  misc_feature (25)..(57)
acaucugaauacgaauguccccaatttaaaaaaaaaaaaaaaaaaaaaaaaaaaaaa

SEQ ID NO: 7 - DNA, 56 bp, Artificial Sequence
  Synthetic Oligonucleotide
  misc_feature (24)..(56)
cuagucggcauaguuuaugguuatttaaaaaaaaaaaaaaaaaaaaaaaaaaaaaa

SEQ ID NO: 8 - DNA, 57 bp, Artificial Sequence
  Synthetic Oligonucleotide
  misc_feature (25)..(57)
aaaaacggccaugcaucaccaucctttaaaaaaaaaaaaaaaaaaaaaaaaaaaaaa

SEQ ID NO: 9 - DNA, 54 bp, Artificial Sequence
  Synthetic Oligonucleotide
  misc_feature (22)..(54)
uaggccaauacccuaccgucctttaaaaaaaaaaaaaaaaaaaaaaaaaaaaaa

SEQ ID NO: 10 - DNA, 56 bp, Artificial Sequence
  Synthetic Oligonucleotide
aaagacuuugauuucucucaaggtttaaaaaaaaaaaaaaaaaaaaaaaaaaaaaa

SEQ ID NO: 11 - DNA, 22 bp, Artificial Sequence
  Synthetic Oligonucleotide
ggauuggguaauuugcgcgccc

SEQ ID NO: 12 - DNA, 28 bp, Artificial Sequence
  Synthetic Oligonucleotide
caagaaagagcuaucaaucugucaaucc

SEQ ID NO: 13 - DNA, 26 bp, Artificial Sequence
  Synthetic Oligonucleotide
cccguguugagucaaauuaagccgca

SEQ ID NO: 14 - DNA, 22 bp, Artificial Sequence
  Synthetic Oligonucleotide
ggguaauuugcgcgccugcugc

SEQ ID NO: 15 - DNA, 26 bp, Artificial Sequence
  Synthetic Oligonucleotide
uuucucaggcucccucuccggaaucg

SEQ ID NO: 16 - DNA, 24 bp, Artificial Sequence
  Synthetic Oligonucleotide
acaucugaauacgaauguccccaa

SEQ ID NO: 17 - DNA, 23 bp, Artificial Sequence
  Synthetic Oligonucleotide
cuagucggcauaguuuaugguua

SEQ ID NO: 18 - DNA, 24 bp, Artificial Sequence
  Synthetic Oligonucleotide
aaaaacggccaugcaucaccaucc

SEQ ID NO: 19 - DNA, 21 bp, Artificial Sequence
  Synthetic Oligonucleotide
uaggccaauacccuaccgucc

SEQ ID NO: 20 - DNA, 23 bp, Artificial Sequence
  Synthetic Oligonucleotide
aaagacuuugauuucucucaagg

SEQ ID NO: 21 - DNA, 15 bp, Artificial Sequence
  Synthetic Oligonucleotide
aatactacagcatgg

SEQ ID NO: 22 - DNA, 19 bp, Artificial Sequence
  Synthetic Oligonucleotide
ggaaggcagcaggcgcgta

SEQ ID NO: 23 - DNA, 16 bp, Artificial Sequence
  Synthetic Oligonucleotide
aatactacagcatgga

SEQ ID NO: 24 - DNA, 17 bp, Artificial Sequence
  Synthetic Oligonucleotide
aatactacagcatggaa

SEQ ID NO: 25 - DNA, 18 bp, Artificial Sequence
  Synthetic Oligonucleotide
atactacagcatggaata

SEQ ID NO: 26 - DNA, 19 bp, Artificial Sequence
  Synthetic Oligonucleotide
attcagatgtcagaggtga

SEQ ID NO: 27 - DNA, 21 bp, Artificial Sequence
  Synthetic Oligonucleotide
gtattcagatgtcagaggtga

SEQ ID NO: 28 - DNA, 18 bp, Artificial Sequence
  Synthetic Oligonucleotide
gttacgattaataggagt

SEQ ID NO: 29 - DNA, 19 bp, Artificial Sequence
  Synthetic Oligonucleotide
gttacgattaataggagta

SEQ ID NO: 30 - DNA, 20 bp, Artificial Sequence
  Synthetic Oligonucleotide
gttacgattaataggagtag

SEQ ID NO: 31 - DNA, 21 bp, Artificial Sequence
  Synthetic Oligonucleotide
gttacgattaataggagtagc

SEQ ID NO: 32 - DNA, 18 bp, Artificial Sequence
  Synthetic Oligonucleotide
aatactacagcatggaat

SEQ ID NO: 33 - DNA, 19 bp, Artificial Sequence
  Synthetic Oligonucleotide
aatactacagcatggaata

SEQ ID NO: 34 - DNA, 16 bp, Artificial Sequence
  Synthetic Oligonucleotide
tacgattaataggagt

SEQ ID NO: 35 - DNA, 17 bp, Artificial Sequence
  Synthetic Oligonucleotide
tactacagcatggaata

SEQ ID NO: 36 - DNA, 20 bp, Artificial Sequence
  Synthetic Oligonucleotide
tattcagatgtcagaggtga

SEQ ID NO: 37 - DNA, 20 bp, Artificial Sequence
  Synthetic Oligonucleotide
  misc_feature (6)..(6): n means a or g or c or t/u, unknown, or other.
tcagtnccttatgagaaatc

SEQ ID NO: 38 - DNA, 16 bp, Artificial Sequence
  Synthetic Oligonucleotide
tggcttagttacgatt

SEQ ID NO: 39 - DNA, 21 bp, Artificial Sequence
  Synthetic Oligonucleotide
tggcttagttacgattaatag

SEQ ID NO: 40 - DNA, 20 bp, Artificial Sequence
  Synthetic Oligonucleotide
ttaataggagtagcttgggg

SEQ ID NO: 41 - DNA, 17 bp, Artificial Sequence
  Synthetic Oligonucleotide
ttacgattaataggagt

SEQ ID NO: 42 - DNA, 18 bp, Artificial Sequence
  Synthetic Oligonucleotide
ttcagatgtcagaggtga

SEQ ID NO: 43 - DNA, 16 bp, Artificial Sequence
  Synthetic Oligonucleotide
ttggcttagttacgat

SEQ ID NO: 44 - DNA, 18 bp, Artificial Sequence
  Synthetic Oligonucleotide
ttggcttagttacgatta

SEQ ID NO: 45 - DNA, 21 bp, Artificial Sequence
  Synthetic Oligonucleotide
ttggggacattcgtattcaga

SEQ ID NO: 46 - DNA, 20 bp, Artificial Sequence
  Synthetic Oligonucleotide
tttagattgcttccttcagt

SEQ ID NO: 47 - DNA, 16 bp, Artificial Sequence
  Synthetic Oligonucleotide
  misc_feature (12)..(12): n means a or g or c or t/u, unknown, or other.
tttgaatactanagca

SEQ ID NO: 48 - DNA, 21 bp, Artificial Sequence
  Synthetic Oligonucleotide
acattcgtattcagatgtcag

SEQ ID NO: 49 - DNA, 20 bp, Artificial Sequence
  Synthetic Oligonucleotide
cttagttacgattaatagga

SEQ ID NO: 50 - DNA, 21 bp, Artificial Sequence
  Synthetic Oligonucleotide
cgattaataggagtagcttgg

SEQ ID NO: 51 - DNA, 24 bp, Artificial Sequence
  Synthetic Oligonucleotide
cttagttacgattaataggagtag

SEQ ID NO: 52 - DNA, 16 bp, Artificial Sequence
  Synthetic Oligonucleotide
  misc_feature (11)..(11): n means a or g or c or t/u, unknown, or other.
cttgaatactncagca

SEQ ID NO: 53 - DNA, 16 bp, Artificial Sequence
  Synthetic Oligonucleotide
ggcttagttacgatta

SEQ ID NO: 54 - DNA, 15 bp, Artificial Sequence
  Synthetic Oligonucleotide
  misc_feature (8)..(8): n means a or g or c or t/u, unknown, or other.
aatactanagcatgg

SEQ ID NO: 55 - DNA, 19 bp, Artificial Sequence
  Synthetic Oligonucleotide
  misc_feature (8)..(8): n means a or g or c or t/u, unknown, or other.
aatactanagcatggaata

SEQ ID NO: 56 - DNA, 17 bp, Artificial Sequence
  Synthetic Oligonucleotide
aattctaaagaagagag

SEQ ID NO: 57 - DNA, 52 bp, Artificial Sequence
  Synthetic Oligonucleotide
  promoter (1)..(27)
aatttaatacgactcactatagggagattcactcccttaactttcgttcttg

SEQ ID NO: 58 - DNA, 51 bp, Artificial Sequence
  Synthetic Oligonucleotide
  promoter (1)..(27)
aatttaatacgactcactatagggagacttgattaatggaagtattttaga

SEQ ID NO: 59 - DNA, 56 bp, Artificial Sequence
  Synthetic Oligonucleotide
  promoter (1)..(27)
aatttaatacgactcactatagggagacttaactttcgttcttgattaatggaagt

SEQ ID NO: 60 - DNA, 47 bp, Artificial Sequence
  Synthetic Oligonucleotide
  promoter (1)..(27)
aatttaatacgactcactatagggagacctactcttgtcttaaacta

SEQ ID NO: 61 - DNA, 53 bp, Artificial Sequence
  Synthetic Oligonucleotide
  promoter (1)..(27)
aatttaatacgactcactatagggagaaaacggccatgcatcaccatccaaga

SEQ ID NO: 62 - DNA, 60 bp, Artificial Sequence
  Synthetic Oligonucleotide
  promoter (1)..(27)
aatttaatacgactcactatagggagactcccttaactttcgttcttgattaatggaagt

SEQ ID NO: 63 - DNA, 54 bp, Artificial Sequence
  Synthetic Oligonucleotide
  promoter (1)..(27)
aatttaatacgactcactatagggagacgacggtatctgatcgtcttcactccc

SEQ ID NO: 64 - DNA, 55 bp, Artificial Sequence
  Synthetic Oligonucleotide
  promoter (1)..(27)
aatttaatacgactcactatagggagacttaactttcgttcttgattaatggaag

SEQ ID NO: 65 - DNA, 57 bp, Artificial Sequence
  Synthetic Oligonucleotide
  promoter (1)..(27)
aatttaatacgactcactatagggagacttaactttcgttcttgattaatggaagta

SEQ ID NO: 66 - DNA, 57 bp, Artificial Sequence
  Synthetic Oligonucleotide
  promoter (1)..(27)
aatttaatacgactcactatagggagacactcccttaactttcgttcttgattaatg

SEQ ID NO: 67 - DNA, 58 bp, Artificial Sequence
  Synthetic Oligonucleotide
  promoter (1)..(27)
aatttaatacgactcactatagggagacactcccttaactttcgttcttgattaatgg

SEQ ID NO: 68 - DNA, 56 bp, Artificial Sequence
  Synthetic Oligonucleotide
  promoter (1)..(27)
aatttaatacgactcactatagggagacttcactcccttaactttcgttcttgatt

SEQ ID NO: 69 - DNA, 55 bp, Artificial Sequence
  Synthetic Oligonucleotide
  promoter (1)..(27)
aatttaatacgactcactatagggagacttcactcccttaactttcgttcttgat

SEQ ID NO: 70 - DNA, 55 bp, Artificial Sequence
  Synthetic Oligonucleotide
  promoter (1)..(27)
aatttaatacgactcactatagggagaatcgtcttcactcccttaactttcgttc

SEQ ID NO: 71 - DNA, 55 bp, Artificial Sequence
  Synthetic Oligonucleotide
  promoter (1)..(27)
aatttaatacgactcactatagggagactcccttaactttcgttcttgattaatg

SEQ ID NO: 72 - DNA, 53 bp, Artificial Sequence
  Synthetic Oligonucleotide
  promoter (1)..(27)
aatttaatacgactcactatagggagatcactcccttaactttcgttcttgat

SEQ ID NO: 73 - DNA, 53 bp, Artificial Sequence
  Synthetic Oligonucleotide
  promoter (1)..(27)
aatttaatacgactcactatagggagacccttaactttcgttcttgattaatg

SEQ ID NO: 74 - DNA, 51 bp, Artificial Sequence
  Synthetic Oligonucleotide
  promoter (1)..(27)
aatttaatacgactcactatagggagacttaactttcgttcttgattaatg

SEQ ID NO: 75 - DNA, 49 bp, Artificial Sequence
  Synthetic Oligonucleotide
  promoter (1)..(27)
aatttaatacgactcactatagggagataactttcgttcttgattaatg

SEQ ID NO: 76 - DNA, 51 bp, Artificial Sequence
  Synthetic Oligonucleotide
  promoter (1)..(27)
aatttaatacgactcactatagggagaactcccttaactttcgttcttgat

SEQ ID NO: 77 - DNA, 49 bp, Artificial Sequence
  Synthetic Oligonucleotide
  promoter (1)..(27)
aatttaatacgactcactatagggagatcccttaactttcgttcttgat

SEQ ID NO: 78 - DNA, 55 bp, Artificial Sequence
  Synthetic Oligonucleotide
  promoter (1)..(27)
  misc_feature (51)..(51): n means a or g or c or t/u, unknown, or other.
aatttaatacgactcactatagggagaaggcaaatgctttcgcagttgttngtct

SEQ ID NO: 79 - DNA, 55 bp, Artificial Sequence
  Synthetic Oligonucleotide
  promoter (1)..(27)
aatttaatacgactcactatagggagaaggcaaatgctttcgcagttgtttgtct

SEQ ID NO: 80 - DNA, 25 bp, Artificial Sequence
  Synthetic Oligonucleotide
ttcactcccttaactttcgttcttg

SEQ ID NO: 81 - DNA, 24 bp, Artificial Sequence
  Synthetic Oligonucleotide
cttgattaatggaagtattttaga

SEQ ID NO: 82 - DNA, 29 bp, Artificial Sequence
  Synthetic Oligonucleotide
cttaactttcgttcttgattaatggaagt

SEQ ID NO: 83 - DNA, 20 bp, Artificial Sequence
  Synthetic Oligonucleotide
cctactcttgtcttaaacta

SEQ ID NO: 84 - DNA, 26 bp, Artificial Sequence
  Synthetic Oligonucleotide
aaacggccatgcatcaccatccaaga

SEQ ID NO: 85 - DNA, 33 bp, Artificial Sequence
  Synthetic Oligonucleotide
ctcccttaactttcgttcttgattaatggaagt

SEQ ID NO: 86 - DNA, 27 bp, Artificial Sequence
  Synthetic Oligonucleotide
cgacggtatctgatcgtcttcactccc

SEQ ID NO: 87 - DNA, 28 bp, Artificial Sequence
  Synthetic Oligonucleotide
cttaactttcgttcttgattaatggaag

SEQ ID NO: 88 - DNA, 30 bp, Artificial Sequence
  Synthetic Oligonucleotide
cttaactttcgttcttgattaatggaagta

SEQ ID NO: 89 - DNA, 30 bp, Artificial Sequence
  Synthetic Oligonucleotide
cactcccttaactttcgttcttgattaatg

SEQ ID NO: 90 - DNA, 31 bp, Artificial Sequence
  Synthetic Oligonucleotide
cactcccttaactttcgttcttgattaatgg

SEQ ID NO: 91 - DNA, 29 bp, Artificial Sequence
  Synthetic Oligonucleotide
cttcactcccttaactttcgttcttgatt

SEQ ID NO: 92 - DNA, 28 bp, Artificial Sequence
  Synthetic Oligonucleotide
cttcactcccttaactttcgttcttgat

SEQ ID NO: 93 - DNA, 28 bp, Artificial Sequence
  Synthetic Oligonucleotide
atcgtcttcactcccttaactttcgttc

SEQ ID NO: 94 - DNA, 28 bp, Artificial Sequence
  Synthetic Oligonucleotide
ctcccttaactttcgttcttgattaatg

SEQ ID NO: 95 - DNA, 26 bp, Artificial Sequence
  Synthetic Oligonucleotide
tcactcccttaactttcgttcttgat

SEQ ID NO: 96 - DNA, 26 bp, Artificial Sequence
  Synthetic Oligonucleotide
cccttaactttcgttcttgattaatg

SEQ ID NO: 97 - DNA, 24 bp, Artificial Sequence
  Synthetic Oligonucleotide
cttaactttcgttcttgattaatg

SEQ ID NO: 98 - DNA, 22 bp, Artificial Sequence
  Synthetic Oligonucleotide
taactttcgttcttgattaatg

SEQ ID NO: 99 - DNA, 24 bp, Artificial Sequence
  Synthetic Oligonucleotide
actcccttaactttcgttcttgat

SEQ ID NO: 100 - DNA, 22 bp, Artificial Sequence
  Synthetic Oligonucleotide
tcccttaactttcgttcttgat

SEQ ID NO: 101 - DNA, 28 bp, Artificial Sequence
  Synthetic Oligonucleotide
  misc_feature (24)..(24): n means a or g or c or t/u, unknown, or other.
aggcaaatgctttcgcagttgttngtct

SEQ ID NO: 102 - DNA, 28 bp, Artificial Sequence
  Synthetic Oligonucleotide
aggcaaatgctttcgcagttgtttgtct

SEQ ID NO: 103 - DNA, 20 bp, Artificial Sequence
  Synthetic Oligonucleotide
cgcgcaagcgagaaagcgcg

SEQ ID NO: 104 - DNA, 22 bp, Artificial Sequence
  Synthetic Oligonucleotide
gcucgcauucgcgcaagcgagc

SEQ ID NO: 105 - DNA, 22 bp, Artificial Sequence
  Synthetic Oligonucleotide
gcuugcgaguauucgcgcaagc

SEQ ID NO: 106 - DNA, 21 bp, Artificial Sequence
  Synthetic Oligonucleotide
ggcaagcgagaaagucuugcc

SEQ ID NO: 107 - DNA, 22 bp, Artificial Sequence
  Synthetic Oligonucleotide
ccgagguauucgcgcaacucgg

SEQ ID NO: 108 - DNA, 23 bp, Artificial Sequence
  Synthetic Oligonucleotide
ggcucacuuucucgcuuggagcc

SEQ ID NO: 109 - DNA, 21 bp, Artificial Sequence
  Synthetic Oligonucleotide
  misc_feature (11)..(11): n means a or g or c or t/u, unknown, or other.
cucuggagacnagcaccagag

SEQ ID NO: 110 - DNA, 18 bp, Artificial Sequence
  Synthetic Oligonucleotide
gucucauuuucuggagac

SEQ ID NO: 111 - DNA, 20 bp, Artificial Sequence
  Synthetic Oligonucleotide
gccuaaaauacuuccuaggc

SEQ ID NO: 112 - DNA, 18 bp, Artificial Sequence
  Synthetic Oligonucleotide
cauggaaauacuuccaug

SEQ ID NO: 113 - DNA, 23 bp, Artificial Sequence
  Synthetic Oligonucleotide
ccgagauuuucuggagaccucgg

SEQ ID NO: 114 - DNA, 25 bp, Artificial Sequence
  Synthetic Oligonucleotide
ccgaggccuaaaauacuucccucgg

SEQ ID NO: 115 - DNA, 19 bp, Artificial Sequence
  Synthetic Oligonucleotide
gggaauuuaaaaccuuccc

SEQ ID NO: 116 - DNA, 21 bp, Artificial Sequence
  Synthetic Oligonucleotide
ggaaggaauuuaaaaccuucc

SEQ ID NO: 117 - DNA, 21 bp, Artificial Sequence
  Synthetic Oligonucleotide
gugggaauuuaaaacccccac

SEQ ID NO: 118 - DNA, 25 bp, Artificial Sequence
  Synthetic Oligonucleotide
uccagaaauucuuagauuuucugga

SEQ ID NO: 119 - DNA, 24 bp, Artificial Sequence
  Synthetic Oligonucleotide
acuccgaacgaaaguuaagggagu

SEQ ID NO: 120 - DNA, 23 bp, Artificial Sequence
  Synthetic Oligonucleotide
agggagugaagacgaucaucccu

SEQ ID NO: 121 - DNA, 23 bp, Artificial Sequence
  Synthetic Oligonucleotide
ucgcgcaagcgagaaaggcgcga

SEQ ID NO: 122 - DNA, 23 bp, Artificial Sequence
  Synthetic Oligonucleotide
  misc_feature (9)..(9): n means a or g or c or t/u, unknown, or other.
ccgaagugncuaaaauacuucgg

SEQ ID NO: 123 - DNA, 20 bp, Artificial Sequence
  Synthetic Oligonucleotide
caccucagaugucagaggug

SEQ ID NO: 124 - DNA, 23 bp, Artificial Sequence
  Synthetic Oligonucleotide
cuaccucuaaagaagagagguag

SEQ ID NO: 125 - DNA, 16 bp, Artificial Sequence
  Synthetic Oligonucleotide
cgcgcaagcgagaaag

SEQ ID NO: 126 - DNA, 16 bp, Artificial Sequence
  Synthetic Oligonucleotide
auucgcgcaagcgagc

SEQ ID NO: 127 - DNA, 16 bp, Artificial Sequence
  Synthetic Oligonucleotide
gaguauucgcgcaagc

SEQ ID NO: 128 - DNA, 15 bp, Artificial Sequence
  Synthetic Oligonucleotide
ggcaagcgagaaagu

SEQ ID NO: 129 - DNA, 12 bp, Artificial Sequence
  Synthetic Oligonucleotide
guauucgcgcaa

SEQ ID NO: 130 - DNA, 13 bp, Artificial Sequence
  Synthetic Oligonucleotide
acuuucucgcuug

SEQ ID NO: 131 - DNA, 15 bp, Artificial Sequence
  Synthetic Oligonucleotide
  misc_feature (11)..(11): n means a or g or c or t/u, unknown, or other.
cucuggagacnagca

SEQ ID NO: 132 - DNA, 13 bp, Artificial Sequence
  Synthetic Oligonucleotide
auuuucuggagac

SEQ ID NO: 133 - DNA, 15 bp, Artificial Sequence
  Synthetic Oligonucleotide
gccuaaaauacuucc

SEQ ID NO: 134 - DNA, 13 bp, Artificial Sequence
  Synthetic Oligonucleotide
aaauacuuccaug

SEQ ID NO: 135 - DNA, 13 bp, Artificial Sequence
  Synthetic Oligonucleotide
auuuucuggagac

SEQ ID NO: 136 - DNA, 13 bp, Artificial Sequence
  Synthetic Oligonucleotide
ccuaaaauacuuc

SEQ ID NO: 137 - DNA, 14 bp, Artificial Sequence
  Synthetic Oligonucleotide
gggaauuuaaaacc

SEQ ID NO: 138 - DNA, 17 bp, Artificial Sequence
  Synthetic Oligonucleotide
ggaauuuaaaaccuucc

SEQ ID NO: 139 - DNA, 16 bp, Artificial Sequence
  Synthetic Oligonucleotide
gugggaauuuaaaacc

SEQ ID NO: 140 - DNA, 21 bp, Artificial Sequence
  Synthetic Oligonucleotide
gaaauucuuagauuuucugga

SEQ ID NO: 141 - DNA, 19 bp, Artificial Sequence
  Synthetic Oligonucleotide
gaacgaaaguuaagggagu

SEQ ID NO: 142 - DNA, 18 bp, Artificial Sequence
  Synthetic Oligonucleotide
agggagugaagacgauca

SEQ ID NO: 143 - DNA, 17 bp, Artificial Sequence
  Synthetic Oligonucleotide
ucgcgcaagcgagaaag

SEQ ID NO: 144 - DNA, 17 bp, Artificial Sequence
  Synthetic Oligonucleotide
  misc_feature (3)..(3): n means a or g or c or t/u, unknown, or other.
ugncuaaaauacuucgg

SEQ ID NO: 145 - DNA, 15 bp, Artificial Sequence
  Synthetic Oligonucleotide
cagaugucagaggug

SEQ ID NO: 146 - DNA, 18 bp, Artificial Sequence
  Synthetic Oligonucleotide
ucuaaagaagagagguag

SEQ ID NO: 147 - DNA, 19 bp, Artificial Sequence
  Synthetic Oligonucleotide
ucuuagauuuucuggagac

SEQ ID NO: 148 - DNA, 15 bp, Artificial Sequence
  Synthetic Oligonucleotide
uucagaugucagagg

SEQ ID NO: 149 - DNA, 16 bp, Artificial Sequence
  Synthetic Oligonucleotide
uucagaugucagaggt

SEQ ID NO: 150 - DNA, 18 bp, Artificial Sequence
  Synthetic Oligonucleotide
uauucagaugucagaggt

SEQ ID NO: 151 - DNA, 19 bp, Artificial Sequence
  Synthetic Oligonucleotide
uauucagaugucagaggug

SEQ ID NO: 152 - DNA, 15 bp, Artificial Sequence
  Synthetic Oligonucleotide
ucagaugucagaggt

SEQ ID NO: 153 - DNA, 16 bp, Artificial Sequence
  Synthetic Oligonucleotide
uucagaugucagaggt

SEQ ID NO: 154 - DNA, 17 bp, Artificial Sequence
  Synthetic Oligonucleotide
auucagaugucagaggt

SEQ ID NO: 155 - DNA, 18 bp, Artificial Sequence
  Synthetic Oligonucleotide
auucagaugucagaggug

SEQ ID NO: 156 - DNA, 17 bp, Artificial Sequence
  Synthetic Oligonucleotide
cuuagauuuucuggaga

SEQ ID NO: 157 - DNA, 18 bp, Artificial Sequence
  Synthetic Oligonucleotide
cuuagauuuucuggagac

SEQ ID NO: 158 - DNA, 20 bp, Artificial Sequence
  Synthetic Oligonucleotide
cuuaguuacgauuaauagga

SEQ ID NO: 159 - DNA, 21 bp, Artificial Sequence
  Synthetic Oligonucleotide
guauucagaugucagagguga

SEQ ID NO: 160 - DNA, 21 bp, Artificial Sequence
  Synthetic Oligonucleotide
auucuuagauuuucuggagac

SEQ ID NO: 161 - DNA, 18 bp, Artificial Sequence
  Synthetic Oligonucleotide
cuaagauuuucuggagac

SEQ ID NO: 162 - DNA, 23 bp, Artificial Sequence
  Synthetic Oligonucleotide
  misc_feature (12)..(12): n means a or g or c or t/u, unknown, or other.
tttgaatactanagcatggaata

SEQ ID NO: 163 - DNA, 10 bp, Artificial Sequence
  Synthetic Oligonucleotide
  misc_feature (6)..(6): n means a or g or c or t/u, unknown, or other.
tactanagca

SEQ ID NO: 164 - DNA, 23 bp, Artificial Sequence
  Synthetic Oligonucleotide
tttgaatactacagcatggaata

SEQ ID NO: 165 - DNA, 10 bp, Artificial Sequence
  Synthetic Oligonucleotide
tactacagca

SEQ ID NO: 166 - DNA, 35 bp, Artificial Sequence
  Synthetic Oligonucleotide
ttggcttagttacgattaataggagtagcttgggg

SEQ ID NO: 167 - DNA, 11 bp, Artificial Sequence
  Synthetic Oligonucleotide
ttaataggagt

SEQ ID NO: 168 - DNA, 14 bp, Artificial Sequence
  Synthetic Oligonucleotide
ggcttagttacgat

SEQ ID NO: 169 - DNA, 63 bp, Artificial Sequence
  Synthetic Oligonucleotide
cgacggtatctgatcgtcttcactcccttaactttcgttcttgattaatggaagtattttaga

SEQ ID NO: 170 - DNA, 51 bp, Artificial Sequence
  Synthetic Oligonucleotide
atcgtcttcactcccttaactttcgttcttgattaatggaagtattttaga

SEQ ID NO: 171 - DNA, 11 bp, Artificial Sequence
  Synthetic Oligonucleotide
cttgattaatg

SEQ ID NO: 172 - DNA, 12 bp, Artificial Sequence
  Synthetic Oligonucleotide
taactttcgttc

SEQ ID NO: 173 - DNA, 10 bp, Artificial Sequence
  Synthetic Oligonucleotide
cttcactccc

SEQ ID NO: 174 - DNA, 14 bp, Artificial Sequence
  Synthetic Oligonucleotide
ucagaugucagagg

SEQ ID NO: 175 - DNA, 17 bp, Artificial Sequence
  Synthetic Oligonucleotide
cuaagauuuucuggaga

SEQ ID NO: 176 - DNA, 13 bp, Artificial Sequence
  Synthetic Oligonucleotide
cagaugucagagg

SEQ ID NO: 177 - DNA, 10 bp, Artificial Sequence
  Synthetic Oligonucleotide
  misc_feature (1)..(1): y means t/u or c
yucuggagac

SEQ ID NO: 178 - DNA, 10 bp, Artificial Sequence
  Synthetic Oligonucleotide
auuuucugga

SEQ ID NO: 179 - DNA, 27 bp, Artificial Sequence
  Synthetic Oligonucleotide
aatttaatacgactcactatagggaga

SEQ ID NO: 180 - DNA, 2087 bp, Plasmodium falciparum
  ref <308>: XR_002273081.2
  ref <309>: 2018-03-28
  ref <313>: (1)..(2087)
aacctggttgatcttgccagtagtcatatgcttgtctcaaagattaagccatgcaagtgaaagtatatatatattttatatgtagaaactgcgaacggctcattaaaacagttatagtctacttgacatttttattataaggataactacggaaaagctgtagctaatacttgctttattatcctttgatttttatctttggataagtatttgttaggccttataagaaaaaagttattaacttaaggaattataacaaagaagtaacacgtaataaatttattttatttagtgtgtatcaatcgagtttctgacctatcagcttttgatgttagggtattggcctaacatggctatgacgggtaacggggaattagagttcgattccggagagggagcctgagaaatagctaccacatctaaggaaggcagcaggcgcgtaaattacccaattctaaagaagagaggtagtgacaagaaataacaatgcaaggccaatttttggttttgtaattggaatggtgggaatttaaaaccttcccagagtaacaattggagggcaagtctggtgccagcagccgcggtaattccagctccaatagcgtatattaaaattgttgcagttaaaacgctcgtagttgaatttcaaagaatcgatattttattgtaactattctaggggaactattttagctttcgctttaatacgcttcctctattattatgttctttaaataacaaagattctttttaaaatccccacttttgcttttgctttttggggattttgttactttgagtaaattagagtgttcaaagcaaacagttaaagcatttactgtgtttgaatactatagcatggaataacaaaattgaacaagctaaaattttttgttcttttttcttattttggcttagttacgattaataggagtagcttggggacattcgtattcagatgtcagaggtgaaattcttagattttctggagacgaacaactgcgaaagcatttgtctaaaatacttccattaatcaagaacgaaagttaagggagtgaagacgatcagataccgtcgtaatcttaaccataaactatgccgactaggtgttggatgaaagtgttaaaaataaaagtcatctttcgaggtgacttttagattgcttccttcagtaccttatgagaaatcaaagtctttgggttctggggcgagtattcgcgcaagcgagaaagttaaaagaattgacggaagggcaccaccaggcgtggagcttgcggcttaatttgactcaacacggggaaactcactagtttaagacaagagtaggattgacagattaatagctctttcttgatttcttggatggtgatgcatggccgtttttagttcgtgaatatgatttgtctggttaattccgataacgaacgagatcttaacctgctaattagcggcgagtacactatattcttatttgaaattgaacataggtaactatacatttattcagtaatcaaattaggatatttttattaaaatatccttttccctgttctactaataatttgttttttactctatttctctcttcttttaagaatgtacttgcttgattgaaaagcttcttagaggaacattgtgtgtctaacacaaggaagtttaaggcaacaacaggtctgtgatgtccttagatgaactaggctgcacgcgtgctacactgatatatataacgagtttttaaaaatatgcttatatttgtatctttgcttatattttgcatacttttcctccgccgaaaggcgtaggtaatctttatcaatatatatcgtgatggggatagattattgcaattattaatcttgaacgaggaatgcctagtaagcatgattcatcagattgtgctgactacgtccctgccctttgtacacaccgcccgtcgctcctaccgattgaaagatatgatgaattgtttggacaagaaaaattgaattatattctttttttttctggaaaaaccgtaaatcctatcttttaaaggaaggagaagtcgtaacaaggtttccgtaggtgaacctgcggaaggatcatta

SEQ ID NO: 181 - DNA, 56 bp, Artificial Sequence
  Synthetic Oligonucleotide
  promoter (1)..(27)
  misc_feature (43)..(43): n means a or g or c or t/u, unknown, or other.
aatttaatacgactcactatagggagatcaagaaagagctatnaatctgtcaatcc

SEQ ID NO: 182 - DNA, 29 bp, Artificial Sequence
  Synthetic Oligonucleotide
  misc_feature (16)..(16): n means a or g or c or t/u, unknown, or other.
tcaagaaagagctatnaatctgtcaatcc

SEQ ID NO: 183 - DNA, 23 bp, Artificial Sequence
  Synthetic Oligonucleotide
gaaatcaaagtctttgggttctg

SEQ ID NO: 184 - DNA, 19 bp, Artificial Sequence
  Synthetic Oligonucleotide
caaagtctttgggttctgg

SEQ ID NO: 185 - DNA, 53 bp, Artificial Sequence
  Synthetic Oligonucleotide
  misc_feature (21)..(21): n means a or g or c or t/u, unknown, or other.
tttagattgcttccttcagtnccttatgagaaatcaaagtctttgggttctgg

SEQ ID NO: 186 - DNA, 24 bp, Artificial Sequence
  Synthetic Oligonucleotide
gaaatcaaagtctttgggttctgg

SEQ ID NO: 187 - DNA, 18 bp, Artificial Sequence
  Synthetic Oligonucleotide
caaagtctttgggttctg

SEQ ID NO: 188 - DNA, 75 bp, Artificial Sequence
  Synthetic Oligonucleotide
  misc_feature (44)..(44): n means a or g or c or t/u, unknown, or other.
aaacggccatgcatcaccatccaagaaatcaagaaagagctatnaatctgtcaatcctactcttgtcttaaacta

SEQ ID NO: 189 - DNA, 24 bp, Artificial Sequence
  Synthetic Oligonucleotide
  misc_feature (10)..(10): s means g or c.
gaguauucgsgcaagcgagaaagu

SEQ ID NO: 190 - DNA, 10 bp, Artificial Sequence
  Synthetic Oligonucleotide
auucgcgcaa

SEQ ID NO: 191 - skipped

SEQ ID NO: 192 - DNA, 1557 bp, Plasmodium vivax
  ref <308>: JQ627153.1
  ref <309>: 2012-08-14
  ref <313>: (1)..(1557)
caaagattacgccatgcaagtgaaagtatatgcatattttatatgtagaaactgcgaacggctcattaaaacagttataatctacttgacattttttctataaggataactacggaaaagctgtagctaatacttgctttagcactcttgattcatttcttgagtgtgtacttgttaagccttttaagaaaaaagttattaacttaaggaattataacaaagaagcgacacgtaatggatccgtccatttttagtgtgtatcaatcgagtttctgacctatcagcttttgatgttagggtattggcctaacatggctatgacgggtaacggggaattagagttcgattccggagagggagcctgagaaatagctaccacatctaaggaaggcagcaggcgcgtaaattacccaattctaaagaagagaggtagtgacaagaaataacaatacaaggccaatctggctttgtaattggaatgatgggaatttaaaaccttcccaaaactcaattggagggcaagtctggtgccagcagccgcggtaattccagctccaatagcgtatattaaaattgttgcagttaaaacgctcgtagttgaatttcaaagaatcgatattttaagcaacgcttctagcttaatccacataactgatacttcgtatcgactttgtgcgcattttgctattatgtgttcttttaattaaaatgattctttttaaggactttctttgcttcggcttggaatcccttgttactttgagtaaattagagtgttcaaagcaaacagatatagcattgcgcgtttgaatactacagcatggaataacaaaattgaacaagtcagaattttgttcttttttcttattttggcttagttacgattaataggagtagcttgggggcatttgtattcagatgtcagaggtgaaattcttagattttctggagacaaacaactgcgaaagcatttgcctaaaatacttccattaatcaagaacgaaagttaagggagtgaagacgatcagataccgtcgtaatcttaaccataaactatgccgactaggctttggatgaaagattttaaaataagaattttctcttcggagtttattcttagattgcttccttcagtgccttatgagaaatcaaagtctttgggttctggggcgagtattcgcgcaagcgagaaagttaaaagaattgacggaagggcaccaccaggcgtggagcttgcggcttaatttgactcaacacgggaaaactcactagtttaagacaagagtaggattgacagattaatagctctttcttgatttcttggatggtgatgcatggccgtttttagttcgtgaatatgatttgtctggttaattccgataacgaacgagatcttaacctgctaattagcggcaaatacgatatattcttacgtgggactgaattcggttgatttgcttactttgaagaaaatattgggatacgtaacagtttccctttcccttttctacttagttcgcttttcatactgtttctttttcgcgtaagaatgtattt

SEQ ID NO: 193 - DNA, 2096 bp, Plasmodium knowlesi
  ref <308>: L07560.1
  ref <309>: 2008-10-02
  ref <313>: (1)..(2096)
aacctggttgatcttgccagtagtcatatgcttgtctcaaagattaagccatgcaagtgaaagtatatgcatattttatatgtagaaactgcgaacggctcattaaaacagttataatctacttgacattttctatataaggataactacggaaaagctgtagctaatacttgctttagcactcttgatttctttcttgagtgtgtacttgttaagccttataagaaaagagttattaacttaaggaattataacaaagaagtaacacgtaatggattcttccatttttagtgtgtatcaatcgagtttctgacctatcagcttttgatgttagggtattggcctaacatggctatgacgggtaacggggaattagagttcgattccggagagggagcctgagaaatagctaccacatctaaggaaggcagcaggcgcgtaaattacccaattctaaagaagagaggtagtgacaagaaataacaatacaaggccaatctggctttgtaattggaatgatgggaatttaaaaccttcccaaaattcaattggagggcaagtctggtgccagcagccgcggtaattccagctccaatagcgtatattaaaattgttgcagttaaaacgctcgtagttgaatttcaaagaatcgatattttaagcaacgcttctagctataaatccacataactgatgcctccgcgtatcgactttgtgcgcattttagctattatgtgttcttttaattaaaatgattctttttaagattcatctattaaaaattcgcttcggcataatttttttgatgatcttgttactttgagtaaattagagtgttcaaagcaaacagatatagcatttgtgcgtttgaatactacagcatggaataacaaaattgaacaagtcagaatttttttgttcttttttcttattttggcttagttacgattaataggagtagcttgggggcatttgtattcagatgtcagaggtgaaattcttagattttctggagacaaacaactgcgaaagcatttgcctaaaatacttccattaatcaagaacgaaagttaagggagtgaagacgatcagataccgtcgtaatcttaaccataaactatgccgactaggctttggatgaaagattttaaaataagagtttttcttttctctccggagattagaactcttagattgcttccttcagtgccttatgagaaatcaaagtctttgggttctggggcgagtattcgcgcaagcgagaaagttaaaagaattgacggaagggcaccaccaggcgtggagcttgcggcttaatttgactcaacacgggaaaactcactagtttaagacaagagtaggattgacagattaatagctctttcttgatttcttggatggtgatgcatggccgtttttagttcgtgaatatgatttgtctggttaattccgataacgaacgagatcttaacctgctaattagcggcaaatacgatatattcttatgtagaattgaatatagtggatttgttagattttgaagaaaatattggaattacgttaaatgtgattcctttcccttttctacttaatttacatttccatctatttcttttttgcgtatgaatgtatttgcttgattgtaaagcttcttagaggaacgatgtgtgtctaacacaaggaagtttaaggcaacaacaggtctgtgatgtccttagatgaactaggctgcacgcgtgctacactgatatgtataacgagttactaaaattacgattttagctgcttgcagtttattttcgtacttttcctccactgaaaagtgtaggtaatctttatcaatacatatcgtgatggggatagattattgcaattattaatcttgaacgaggaatgcctagtaagcatgattcatcagattgtgctgactacgtccctgccctttgtacacaccgcccgtcgctcctaccgattgaaagatatgatgaattgtttggacaagaaaaaattggattatatctttttttttggaaaaaccgtaaatcctatcttttaaaggaaggagaagtcgtaacaaggtttccgtaggtgaattc

SEQ ID NO: 194 - DNA, 2091 bp, Plasmodium ovale
  ref <308>: AB182491.1
  ref <309>: 2007-07-24
  ref <313>: (1)..(2091)
aacctggttgatcttgccagtagtcatatgcttgtctcaaagattaagccatgcaagtgaaagtatatgcatattttatatgtagaaactgcgaacggctcattaaaacagttataatctacttgacatttctacttacaaggataactacggaaaagctgtagctaatacttgctttaatacgtttgattcatttttgtctcttacgtatgtacttgttaagcctttaagagaaaagtttacaacttaaggaattataacaaagaagtaacacataataagtttaccttatttagtgtgtatcaatcgagtttctgacctatcagcttttgatgttagggtattggcctaacatggctatgacgggtaacggggaattagagttcgattccggagagggagcctgagaaatagctaccacatctaaggaaggcagcaggcgcgtaaattacccaattctaaagaagagaggtagtgacaagaaataacaatacaaggccatttcatggttttgtaattggaatgatgggaatttaaaaccttcccaaaattcaattggagggcaagtctggtgccagcagccgcggtaattccagctccaatagcgtatattaaaattgttgcagttaaaacgctcgtagttgaatttcaaagaatcaatattttaagtaatgcttttggtataagatgcttaggcaatacaacgtatctgctctttgcattccttatccaaaatgtgttcttattataaaaaggattctttttaaaatctcctttactttttgtactggagattttgttactttgagtaaattagagtgttcaaagcaaacagttaaagcattttactgcgtttgaatactacagcatggaataacaaaattgaacaagtcaaaactctgttcttttttcttattttggcttagttacgattaataggagtagcttgggggcatttggattcagatgtcagaggtgaaattcttagattttctggagacaaacaactgcgaaagcatttgcctaaaatacttccattaatcaagaacgaaagttaagggagtgaagacgatcagataccgtcgtaatcttaaccataaactatgccgactaggttttggatgaaagatttttaaataagaaaattccttttggaaatttcttagattgcttccttcagtaccttatgagaaatcaaagtctttgggttctggggcgagtattcgcgcaagcgagaaagttaaaagaattgacggaagggcaccaccaggcgtggagcttgcggcttaatttgactcaacacggggaaactcactagtttaagacaagagtaggattgacagattaatagctctttcttgatttcttggatggtgatgcatggccgtttttagttcgtgaatatgatttgtctggttaattccgataacgaacgagatcttaacctgctaattagcggcgaatacgttatattcctacttgaaattgaatatagctgaatttgcttattttgaagaatatattaggatacattatagtgtccttttcccttttctacttaattcgctattcatgctgtttcttttttgtgtaggaatgtattcgtttgattgtaaagcttcttagaggaacgatgtgtgtctaacacaaggaagtttaaggcaacaacaggtctgtgatgtccttagatgaactaggctgcacgcgtgctacactgatatgtataacgagttactaaaaatatacttttgtttgagtatttatactctctcaaatagtatacttttcctccgccgaaaggtgtaggtaatctttatcagtacatatcgtgatggggatagattattgcaattattaatcttgaacgaggaatgcctagtaagcatgattcatcagattgtgctgactacgtccctgccctttgtacacaccgcccgtcgctcctaccgattgaaagatatgatgaattgtttggacaagaaaagggaaaattatattttcttttttctggaaaaaccgtaaatcctatcttttaaaggaaggagaagtcgtaacaaggtttccgtaggtgaacctgcggaaggatcatta

SEQ ID NO: 195 - DNA, 2152 bp, Plasmodium malariae
  ref <308>: AF487999.1
  ref <309>: 2002-05-06
  ref <313>: (1)..(2152)
aacctggttgatcttgccagtagtcatatgcttgtctcaaagattaagccatgcaagtgaaagtatatgcatattttatatgtagaaactgcgaacggctcattaaaacagttatagtctacttgacattttttttataaggataactacggaaaagctgtagctaatacttgctttaatactcttaattctttatgttttttgagtatgtatttgttaagccttataagagaaaagtatattaacttaaggaatataacaaagaagtaacacataataaatttcgatttatttagtgtgtatcaatcgagtttctgacctatcagcttttgatgttagggtattggcctaacatggctatgacgggtaacggggaattagagttcgattccggagagggagcctgagaaatagctaccacatctaaggaaggcagcaggcgcgtaaattacccaattctaaagaagagaggtagtgacaagaaataacaatgcaaggccaaattttggttttgcaattggaatgatgggaatttaaaaccttcccagaaggcaattggagggcaagtctggtgccagcagccgcggtaattccagctccaatagcgtatattaaaattgttgcagttaaaacgctcgtagttgaatttcaaggaatcaatattttaagtaatgctttgtatatttataacaaagttgtacattaagaataaacgccaagcgttatattttttctgttacattttgttttattaatatatatatgcgttcttattataaaaatgattctttttaaaattcttttgtataattttttatgcatgggaattttgttactttgagtaaattagagtgttcaaagcaaacagttaaaacagtttctgtgtttgaatactacagcatggaataacaaaattgaacaagtcagaattttgttcttttttcttattttggcttagttacgattaataggagtagcttgggggcatttgtattcagatgtcagaggtgaaattcttagattttctggagacaagcaactgcgaaagcatttgcctaaaatacttccattaatcaagaacgaaagttaagggagtgaagacgatcagataccgtcgtaatcttaaccataaactatgccgactaggtgttggatgatagagtaaaaaataaaagagacattcatatgagtgtttcttttagatagcttccttcagtaccttatgagaaatcaaagtctttgggttctggggcgagtattcgcgcaagcgagaaagttaaaagaattgacggaagggcaccaccaggcgtggagcttgcggcttaatttgactcaacacggggaaactcactagtttaagacaagagtaggattgacagattaatagctctttcttgatttcttggatggtgatgcatggccgtttttagttcgtgaatatgatttgtctggttaattccgataacgaacgagatcttaacctgctaattagcggtaaatacactatattcttaagtgaaattagaatatagataaattgtgctaattttgattaaaatattagaatgttttttttaataaaaacgttcttttccctttttttcttaattatgcatatttattctttttcttttttcgcataagaatgtatttgcttaattgtaaagcttcttagaggaacgatgtgtgtctaacacaaggaagtttaaggcaacaacaggtctgtgatgtccttagatgaactaggctgcacgcgtgctacactgatatgtataacgagtatttaaaaatatatatcttgttatgttatatgtatttctatatgtatgcatgcaaagaatatatagttttcctccactgaaaagtgtaggtaatctttttcaatacatatcgtgatggggatagattattgcaattattaatcttgaacgaggaatgcctagtaagcatgattcatcagattgtgctgactacgtccctgccctttgtacacaccgcccgtcgctcctaccgattgaaagatatgatgaattgtttggacaaggaaaaagggtttttttcttttttctggaaaaatcgtaaatcctatcttttaaaggaaggagaaagtcgtaacaaggtttccgtcggtgaacctgcggaaggatcatta

SEQ ID NO: 196 - DNA, 48 bp, Artificial Sequence
  Synthetic Oligonucleotide
  misc_feature (34)..(34): y means t/u or c.
  misc_feature (44)..(44): n means a or g or c or t/u, unknown, or other.
guauucagaugucagaggugaaauucuuagauuyucuggagacnagca

SEQ ID NO: 197 - DNA, 43 bp, Artificial Sequence
  Synthetic Oligonucleotide
guauucagaugucagaggugaaauucuuagauuuucuggagac